European Patent Specification EP 4 172 170 B1, published September 25, 2024. Title: Fluorescent Cytosine Analogues and Their Application in Transcription and Translation. Applicant: Chalmers Ventures. The sequence listing filed with the application follows.

SEQUENCE LISTING (2 sequences)

SEQ ID NO: 1 - DNA, 20 bp, Artificial Sequence
  DNA Primer
gaagtgccattccgcctgac

SEQ ID NO: 2 - DNA, 20 bp, Artificial Sequence
  DNA Primer
cactgagcctccacctagcc